European Patent Specification EP 3 600 372 B1, published May 13, 2026. Title: SYNTHEKINE COMPOSITIONS AND METHODS OF USE. Applicant: The Board of Trustees-Leland Stanfod Junior University Garcia, Kenan C Gonzalez, Ignacio M. The sequence listing filed with the application follows.

SEQUENCE LISTING (2 sequences)

SEQ ID NO: 1 - protein, 351 aa, Artificial sequence
  synthetic polypeptide
ARGCHIAQFKSLSPAELQAFKRAKDALEESLLLKDCKCRSRLFPRTWDLRQLQVRERPVALEAELALTLKVLEATADTDPALGDVLDAPLATLHHILSQLRACIQPQPTAGPRTRGRLHRWLHRLQEAPKKESPGCLEASVTFNLFRLLARDLNCVASGDLCEGSGSGLGCDLPQNHGLLSANTLVLLHQMRRISPFLCAKDARDFRFPQEMVKGSQLQKAHVMSVLHEMLQQIFSLFHTERSSAAWNMTLLDQLHTGLHQQLQHLETCLLQVVGEGESAGAISSPALTLRRYFQGIRVYLKEKKYSDCAWEVVRMEIMASLFLSTNMQERLRSKDRDLGSSAAAHHHHHH

SEQ ID NO: 2 - protein, 313 aa, Artificial sequence
  synthetic polypeptide
MKTIIALSYIFCLVFAGSHIHGCDKNHLREIIGILNEVTGEGTPCTEMDVPNVLTATKNTTESELVCRASKVLRIFYLKHGKTPCLKKNSSVLMELQRLFRAFRCLDSSISCTMNESKSTSLKDFLESLKSIMDMDDSGSGSGINYKQLQLQERTNIAKCQELLEQLNGKINATYAADFKIPMEMTEKMQKSYTAFAIQEMLQNVFLVFRNNFSSTGWNETIVVRLLDELHQQTVFLKTVLEEKQEERLTWEMSSTALHLKSYYWRVQRYLKLMKYNSYAWMVVRAEIFANFLIIRRLTRNFQNAAAHHHHHH